European Patent Application EP 4 137 156 A1, published February 22, 2023. Title: AGENT FOR PREVENTING OR TREATING AT LEAST ONE CANCER SELECTED FROM THE GROUP CONSISTING OF PANCREATIC CANCER, LUNG CANCER, COLORECTAL CANCER, BILE DUCT CANCER, AND LIVER CANCER, COMBINATION DRUG COMPRISING THE AGENT, AND METHOD OF SCREENING AGENT FOR PREVENTING OR TREATING CANCER. Applicant: THE UNIVERSITY OF TOKYO TAK-Circulator Co., Ltd. The sequence listing filed with the application follows.

SEQUENCE LISTING (10 sequences)

SEQ ID NO: 1 - DNA, 3532 bp, Human
tcaagaggcggggaggagaggaggaaaaagcgctgagtgagggcgggcgggcgggcgggagggagggagtggaggagccggggaggggctccttaaagaaacgcttctgtcgctcgcctgctcgcttttcgctcggcattgcggccagccagccgggcactcggggggcacgcgcggccaccgctagagctctgcccccaccccacccgccagcaggtctggggtggggacccaggtgggggctcctgcagccactgcccggtgcggaccgcacggagcgacccactcctcccagcaccgaggaagaagcaacggagccctcagcaggcgaccggcctccccgcccctgaccacccgcttcccggctgcctttgtggccgcagcttctcgccgccgagccgagggccggcgggggcgcggcgcgcacggccgagcgatgcccagctcgctgttcgcagacctggagcgcaacggcagcggcggcggcggcggcggcagcagcggagggggagagaccctggatgaccaaagagccctgcagctcgcgctcgaccagctctccctgctggggctggacagtgacgagggcgcctctctgtacgacagcgagccgcgcaagaagagcgtgaacatgaccgagtgcgtgccagtacccagttctgagcatgtcgccgagatcgtggggcggcaaggttgtaaaatcaaagcgctgcgggcgaagaccaatacttacatcaagaccccagttcgcggggaggagcctgtctttgttgtgacgggcaggaaggaggatgtggccatggctcggagggagatcatctctgctgccgagcacttctccatgatccgcgcctcccggaataagaacacggcactcaacggcgcggtgcctgggccgcccaacctgcccgggcagaccaccatccaagtgcgggtaccctaccgcgtggtggggctcgtggtggggcccaaaggcgccacaatcaagcgcatccagcagcagacgcacacgtacatcgtgacgcccagccgggataaggagccggtgttcgaggtgaccggcatgccagagaacgtggatcgcgctcgagaggagattgaggcgcacattgctctgcgtaccggcggcatcattgagctcacagacgagaacgacttccacgccaacggcaccgatgtgggcttcgatctgcatcatgggtccggcgggtccggcccaggcagcctctggagcaagcccacccccagcatcacgcccacccccggccgcaagcctttctctagctaccgcaacgacagctccagctcgcttggcagtgcttccacagactcttatttcggcggcgggaccagcagcagcgcagcggctacccagcgcctggcggactacagcccccctagccccgccctgagctttgcgcacaacggaaacaataacaataacggcaatgggtacacctacacagcggggggagaagcctcagtgccatcccccgacggctgccccgagctgcagcccacttttgacccggctcccgctcccccacctggggcaccacttatctgggcccagttcgagcggtccccgggaggcggacctgcagctccggtatcttcttcctgctcttcttctgcatcttcgtctgcttcttcctcctccgtggtcttccccgggggtggcgccagtgcgccctccaacgccaacctggggctattggtgcaccgccggctgcaccctggcaccagctgcccgcgcctgtctccacccttgcacatggccccgggggcgggagagcaccacctggctcgccgggtgcgcagcgacccgggtggaggaggcctggcctacgccgcttatgccaacgggctgggggcacagctgcctggcttgcagccgtcggacacgtcgggctcctcctcttcgtccagctcctcctccagctcttcatcctcttcctccgggcttcggcgtaaaggcagccgcgactgctccgtgtgcttcgagagcgaagtgattgccgcgctggtgccctgtggccacaacctcttctgcatggagtgcgccaatcgcatctgtgagaagagcgagcccgagtgcccggtctgccacaccgcggtcactcaggccatccgcatcttttcttaaaggcagcgggcgctgctagtgcgcaccgtgctgggggaagggggaacccctccccatcctctttccccagcgctcgcctgcctccctgggtgccccccctctcccttctccttcccggccccaccaacactctgagatccgagaggagcttggaaagctgtagtatccgctcatttttaaaatttaatttttaagtaaaggaatttgccaggatatctgcatcaagagtactgtagcctgggaaacctgaacacctgaaatgcatgctctataaataataggaacggcgacattctagtaatgatagtttttacactgtacttaataggaagcttccaaaagaagaaaaccccacaagttttccattttcttaaagtaggaaaaaatgaacagtaataattatgatgaagatgatagtagtgctatgggatgtgtggactgtttagtgtgttcccctttgtgggtgggttcctatgatacttattatagaacacagtggatcctttttgaatgttcgtggaagggccaggagttcctgtgaaaccaggatactgcagctttattaaagttaaagaaactgtaacatatctcttatatattaaaaacgtttaaaagttttaaagagaaattgcattaatacagattgaagtattttattcttttttgacttgaaaaattatatttcatattgcaaagatgtttacaagtattttaatttaagttcagtgaacttttttgtagctgggttaaatctttttattttagtatggccttatggcaaagaacactgtattattttaataatcacacaattgtgacggaattacaaccataaaatgtgtaatgttttgaacagtattctgttgggatggagattttataggttcagacaaatcttctagatctgcttcacccagcatattttctattcagtgatataaagcatattttattctatattattacaaaaacggaaatgtataaacatgtcaaaaagaactgttgatgctttctaacatttgtataaatagaattcagtgcaagttacaaaaattctgttgcaccactctagttttagtatttctattttaatacatttgtttaccacttgtttatgtatatgtaggtgatgttacttgagcttaaatgtactttactgagcaaagtttaaaaaacaaagtatattttattttatgataaagggcctttaacctcatggtcaaatactaatattatatttgctgagacaagatttgaaattgtatcaagagttttatttttctgacatttaaagttctacataataaaggtaaaacttaagtaatggtgctacttcattttttaagtatttctatataaataaaatattgaagaaaatcttaaaaa

SEQ ID NO: 2 - DNA, 35919 bp, Human
ctccaggtgtgttactgaataacaacaacaataatggaatagtttgaaatgccaggcacagtctgaagtgtgttatagacttgtattatctcactcaagcctcacagcatccctgcgtgaaggtggaatcattatcccaaatttgcagacaagactgaggctcagagagatcagtaagtagtagagctgagattcaagcctggattcgcttgactccgtagtccatgtactaactaaccactaggttaaactcccttgttgggcctgacccatgaattggaaaaccagaacctggccccatcttcgtcagtacttggctgggtcaccttgagaaagtcactttccctctcctgtcctctgatttattatgagtcaaatacaggtagtacctatcagggtttcctgaagaggtacctatgaaaatgatttgtttccctgctgtaagtgataagaaaacctccaaagataatgcccccctgtctttttaaggcttctcattctttcttatggcactttctgctcatgagtggaaacttatgtgtatttactgcagggacaaccacattttgtccgcagagctatggggtgcagcaaaggaaggtaggatttggtacatttccccaactctctcctgaccagatccatatattctcagctggttggaggcgtgactccaatctaactgacccacaaaacctctgcctctctcccttctctgcttgactcatccattcttcagaacccagtttgggagatctcttccagaaaggcttctgtgaccatcagtctgagtgtggggcttctccttgagctcccaccaagctctctctcttttttttttcttttttccacacaggattgtgctctgtcactcaggctggagtccagtggtgcgatcatagctcactgcagccttgatctcctgggctgaagtgatctttccacctcagcctcccaagcagttgggaccacaggcatgcatcatcacgcctggctaattaaaaattttttttttcagagaaggggtcttgctatgttgtccaggctggtcttaaactcctgggctcaagcgatcctcccgccttggcctcccctagtactggggttacaggcatgagggactgagctgggcaccacgctctccttgtaacttcttcctctctccacaaaggcagggactttgattgtctaatgcctgatctgctgcccagcaggaacgctctcagtaaaagatgaatgaatgaaaaatgggtcagatgcacctgcaatgatgtgtgattcattctcaaagttgtgtgggtgtctggttggactctgctcatgttcctcctgtgtccccaggtcccacttctcactgatgcgccccaggcagtctgtggtgctctactctttctccagggccacctatcactgaacctacaggatggccctgatgaatcaggggcaggtggcacaggtggatggcaggggtacaatgtgccagaagtgaggtgttcaccccctgttcaggtggtttgggttggagtctaagctggtttcctctattcctgtcttactcaagggaaattcctacccctggccaagacagaaataggagaaaccagcttaaaatccatccctttcctctgagacagaaaaccatcaaagtgtaacacattcaccttatctaaggaaacctcaaatttactcaaaatggcagagagagaaaaatgcgtctcttgtgtgtgtggagttggagccacataatgcacattcagagggtttacacccctcatggaggattcttctccttataaagttgccacaaaagaagagacacagccatggatgctcacaacctaactaagattaggataagcctatggggcggggcggtggggcagacagacaggaatacaatgccttctgcctctgcatgccatttgtctttcagggaaatctggctgagaactgctgtagatacttgctatcagcaagacactctcccatttcctaccccagagttatgaggagtgtacgtgctgctggatgggagcagcgcctgggcagattccatagacagaaatgtgattctgatggaaataaaacaaacaaacaaagcaaactcagcaaaagtctcagcagtcatgaaccttctgggaaagagctgcactaaattaccgagtctcttcatttagatgaaagtgcgtgtcttgagacatcattgttattttaaccatctgggaggaaagtattctccctaaagcctgagctccttgaaggcagagctgtgtcttacataactctacatcatccatggcgcctggttgtagtagttgccttcccaatacctcttcttttcttctttaccaacagaacctctgtattgttggggtttgaagtaataagctacatttcccattcttcttgcacagagagatggcaaatgagatgtaagcaaaattgattaaagcgctgttagagctgtttgaaagggattgagaagaatgcctttttgctgtttccctttcctcctgcctgctgactggaatttacatgtgatgacttgtatttcagcagccattttgtgattatgagttgactttgaagatgaaagccacatgctataagaatggtgaagcaaaaagataggtttctaaagcttctgaacagcaaaggaaacaatcaaatgtaccccataaatatatacacctattatatgcccataataattaaaaaattaaaaaggggctgggagcagtggctcagacctataatcccagcactttgggaggccaaggcaggtggactgctgagctcgggagtttgagatcagcctgggcaacacggtgaaaccctgtctctaaaaaaaaaaaaaaaaaaaaaaattagctgggagtggtgtgtgcctgtgttcccagctactcaggaggctgaggtgggaggattgcttgagcccaggaggttgaggctgcagtgagccatgataacgttactgcactccagcctgggcctgttatgcaaaagtgcatgggctctgggagagaggttgggaggctcgcctttgaatatgggtattaagcttcagtggatgaattatatatcatttattaatatcttggctgctcagaaacctttttactcacttgcagctttggccacatcttaaacagctgcatagctagctctaaacaggtgagaattctgaacactacatctcaaatttcctttttttttttttttgagacagattcagattcttgctctgtcacccaggctggggtgcagtggcacggtcttggctccctgcaacctccgcctcccgggttcaagcgattctcctgcctcagcctccccagtagctaggattacaggcgcatgccaccacgctcggctacttttggtatttttagcagagacggtgtttcactatgttggccaggctggtctggaactcctggccttgtgatctgcccacctcggcctcccaaagtgctgggattacaggtgtgacccaccacgcccagccacatttcaaatttctaagagctcaggcacagggaggtgagcatgacatcaggtaagggaagtaagggttcggtctgtcgttcctgctggacactgaaggtggacgtgtatttgatgaccagatagaagatgggtccttgtgtagtcttttcacttcagaggagttcctttgctctcttggggcttcgggttccctttccatccagatgcccagatgctcctagactggttcttccctttcttccctggctttctgttttctgtgcttgctcaggggaatagtgtgggaagacagtttccctcacaggttcaaggcggtagagcgttgttgagggtctcctgctggagaagtggaactttgcgactgtcactcaggagtgcaatgcagtttctgagatgaaaatttgcgaaccaatttcacgtggtcaatgttgtgaatgaatttatagctagtgaggctctgagtgctgatcagctgggatgactttggagctagatctgaatactaatgggactgggtgactttagttggtgagaattttgagaccctctttgttttgtttaaaatggtctgaggcttttttttttttttttttttttttgagatggagtcttgctctgtcgcccaggctagagtcagtggtgtgatctcggcttaccgcaacctccgcctcccaggttcaagcgattctcctgcctcagcctgctgagtagctgggactacaggcgcctgccaccacgcccaggcaatttttggatttttagcagagacggtgtttcaccatgatggccaggctggtctggaactcctgaccttgtgatctgcccacctcggcctcccaaagtgctgagattacagccatgtgccaccacacccaggcgtattatatcaataacaatttcttagttttgacaaatgtaccatgattgtgtaagatgttactagtaggcaatgctggataaagggtatacaagaatcatatatgccatctttgtaactcttctgtaaatctaaaattattccaaaattaaaagtttaaaataatttttaaaaagtcaatcaccaaaaagtaagtacatttaggacatagatacatgcaagacatgtgtaacataactgaaaatcacagattttggagtcggacgtacctggtttctcatcctggctgccccaattgctaactgcaatgttgggcaaatttctttattccttcaagctctgtgttccaatctctaaaataggaatcctaattatatatacttcaaggggttcctgggaagagtaaatgagaaaatactggcaaagtgccttatcatagtgcctgattgcctgatacatagtaagagctcaataaaagtagcttttattattcttgcaggtgatcaaagaaatgcagagtcaaacaatgttggcaaatgatttcacacctactgaatcggcaacaactgtgatccccagtgcctgacagagtgtgctgaaaccggtacattcataaactgtaaaccagtacagctatttggaaaagcaacgtagcaatatagacacagcaagagactgcagaaatggtcacaacctttcgcccagacctcctcttaatgatttgcagggttccaggcaagggtataaatggagcctcacataccatatgtataagtagtttaaagttagaaatcaggttacaaactgttaaatgaaaatatgttctagcctcctgccttggcaaatatactgtcaccaccacctggaagggctcaagttaaaaattctcagatgcctctgcatcctgtgttggaacatgacggcatggggagagccagttgctagcccccagacccactgtctttccaattcctaagtctgtccagcactgagggggcctcatgtgaatgtgagtggacagcctagcccatgcgtccaaactctgttcactaccccctgcctgtggccactcctcagatccgggtgtgtctactggtggtgtgattggatctcaggaggagagactcagggaccagggctgggcaggccctggagatgagcatggggccagtgggcagggacttctgggagtcctaggcacctggagaatggtctaaaagggaggacgtggatttgcaatgggcatgttcccttggcctgcagactcctcaccaggtgggagggacgcagcccaaggagggccagggggacaccccctgcctgatctcactgcagtactccttagagtccatccaaaggaaagaaatagttcagcagaataaaaaggctacgggcacaaagatagtatcactgtgttgcatttgacactaaaaaaacccaatctaatgttcaacagtagggaaatgttaagacaacaatgataaagctattcagagaagtagtatgctaccaccaacactggcacatgtgacaaccatgtcataacatgggataatgtttatgtgtagatataatagtaaatgaactctggcaactgtgcaaacatctgtgcgccctaggtgagatgcggaagtcaacctgcagacatgagaacagctgcctcaaagagggttgaactctttcaggcagctgaaagattttcctcccaaaattgtctctttcctgtggctggggagaagcagggacttttcaggaactaatgggtaagagctggctggttagactggagttttttgtgcaactctactcaggagttggagataagaacctgctacctgctgcatggaagccagaaaagcactttagctaatcacactccctctctgcgtgggctgaagatatccttgagtcctcccagccctgagcccttctccaggggccagcacacccagaaaccacgcgtgcagtgtttgctctggatgcccaggatagtctctgctgcgcgtgtgaagctctgccatgggctgggtatggaacgggccatgtcacactgagtcctcgcaacaacctggtgagatgggagcctcagcatggctgacttggacactgagatgctggtccagcaccacgcagttggcaagcagagaagccagcctttgaaactctgtgcttccatttgggcacgtacactgggaaatcaaaaggcagtgttccctttctccccacaaactgcttctagtgtcccatggggccagaggaactcaatcaaaacaatattccatagatgtgggatagtggtagcacaaataaattaacaattgcacttctgggcactcgactgtccccacggttctaaaaatgaaaagactctggtatttaatttatattttataagagtgaaaaaggccaggcacagtagctcacacctttaatcccatcattttggaaggccaaggtgggaggattgcttgaactcaagagttcaagaccagcctgggcaatatggcaaaactctacaaaaaaattagccgggtgtggtggtgcatgcctatagttccagctactcagagactgaggtgggaggatcacttgagcctgggaggtcgagactgcagtgcgccaagatagcaccactgtacttcagcctgggaaacagtgagattctgtctcaaaaaaaaaaaaaaaaaaaaaaaaatttgataattgcctttggtaaggaagagctgattttagcatggaacagagggtggcaaacaacagccttcaagccaaatctattccactgcttgtttttatatgtcccatgatctaaataatgggttttacatttttaaatggttggtggggggaaatgtgaaacttacatgaaattccagtctccagatctataaataaagttttattggaacacagccacattcagttgtgcatatgtattgtctacggcagcttctgcactataccagcagagttgaggagttgtaacagggagatcatatggcctgaaaagctgaaaaattttactatctggtcttttacagaaagactttgctgacccctgaaatggaagaagactacaggcctagttatttagtgataattgaacccagctttcattgtttgagtagcttctgcatgtcgattgttaagctttacttacctagattacttcaaatcctacaaagtacatattatcgatcccctgagcaaagctaggatattagctgaagccttaaattcaaattcttactttttaaatttaatttaatttaattaaaattttttttttagagacagggtctcgagctctgttgcccaggctggagtcagtggcatgatcatagctcactgcagcctcaaattcctgggctcatgtgatcctcctgccttggcctcccgaagcactgggattacagtgcctggtctcaaattcttacttccataccatggcagaggagcagagcaagacctcttcagaaacatgagctctaaccaaggcagggaaaatatatttagaggtcctgaatactgaaaacattacagtgtaccttccccagccacccctctgtataatccaaaatattaaacattgttgaactcaaaactgagtgaaagcaagtccaacagagttctaattccctccatgataactacatgtttttctaaaatagtatccgactattttatgagaattttttggtgtccctaggtatatacttgcttcatttgttgggtgattaaaccccaaaactgaccaaaatctgttggccttgctaagtctgagctcagggcacagaagaagagtctcacattgtgacagccacctggcgtggcgatagagtcctgttctttccaccaagagagaagccgtccctagagaagtctctcatttaagaaagcagaacatatctactcaaaaagccatggggccacctgaatcaaatgcctgtcagaccttctccctcacctcaggtctgtgtctccctaagcccatgtcatgatcagagatgttccttaaagctgggctccccagcccccaggccatgcaccagtacaggtctgtggcctgttacgaacaggaggtgagtggcaggtaagcaagcattactgatggtaatggcaggtcatctggagtgtctgctgccatcatactggctgcagcaggaatgcgcaagtggggctgtgtgctccatgaagccagcgggaaccagggacaagtgggagctccacctcttccgagttggggctggagctccctgggtgccacttcagctgcccaaatggcagctgcagacccaggcctcttgcagatgggagccccgccctcccaggcatagcaggcagacaagttcctgggcagaaggaggtgggtcctggtgaggccccaccttcaggccagggagggtctgaagtctgtgggcccagctgccagtctggtgaaccagagtggggacttgtgctgccttttttgggctcatccatggccactcattggaccaatcagtacatacttcctcccctctgaggcccataaaagccctgggctcagccagagcagaggaaaggacggagagacactgggatagccagctgcagagagaagataacctctcatcagggaactacagaggacaggacaaccagcctgcagagaggagctaccctctctgctaggagctaaacacttgtcaggacaccctagctacagaggagctgcccactgcaagtcttctttgagctgttctattgctcagtaaagctcctcttcatcttgctcaccctccacttgtccacataccttattcttccatgttgcaggacaagaactcgggacccactgaatggtgaggctaaaagagctgctgtaacacaaacagggctgaaacatgccccttgcttgccacattgtgggtgaagagaaggagagaagagctgcagcccttcagggatcccagacctgggagctccctgagccagagccgtgactccctctttggggttctgtggttcctggcatctgcaagcttctgggtgccactgcattccccagtgccagccagggaagtggcttgcagtgcacctggtccagccacaaccttgcagagagcgctgctggcacctgtagctgcctgccccacagcagccaccagtatgtctgactgagcagtggccggaccccatgctcgctcacacacccctcactgttccacacccgactcacccttggcaggcgtgggacccaggccagcagtgtgaactgagtacagcctgccaggcccagcaggcctgagcaaaacttgggtaaaaacatcactggccacagaggtttctggctaggaaaacaacaccccaaggatcctgtaacattcatcggaacgccacctcccgttagatcagcggtggcatgagattgtcataggagcacaagccctattgtgaactgtgcgtctaagggatctaggttgtgtgttccttataagaatctaagatcgctgagattgatgagatcacttgagcccaggagtttgagaccagccttggtaacacggtgaaaccccatctttaccacaaaaacaaaaattagctggatgtggtggcgtgtgcctgcagtcccagctacagggactgaggtgggaggatcacttgagcccagggaggttgaggctgcagtgagctgagattgcaccactgcactccagcctgggtggcagagtaagaccttatctcaaaaaacaaaaccaaaatggtttattgtaaaaaaaatgagtatggtcaatatttttttctcctcagttctactttaatttcaagcactcaagtgaggatcaagcatctgatgagaatgggagagaaaggcagagagagctgtgtctgttcaggaaaccgcatcctttcacaattagggaaacaacaatttttttttgaggcagggtcttgctctgttgcccagggtgaagggcagtggcacaaatcatagctcactgcagcctcgacctcccgggttcaagcaatccccttacctcagtctctcaagtagctgggactacacacatgcaccatcacgtctggctaatttattttcatttttaattttttagtagaaacagggtctctccagaaaaactacagatggatcagacaattaaatactgaaccctgtggaacaaatagaagagaaagtgaaggcttgtctatccctagacacactctttctggaacatccgtcttcctcacactgtcccctcttgacttccatgataccctaggctgctggtttttctcctacctctctggccagtctttctcagtcttcttggccggctccccctgtttctgagccccaatccctatatgttggagtccttttgggtctcaatttttttttactccttctcttttagggttttcttcctatgagatctttcagtctctagcctttaatgccactgagtgttgccatttctactcccatgttcataattccagccctgatgtctggcctgacacttagagactgtccacggagggatacaggaacaaaggaagtgacaggagtgacaaaggaaaagatgcgtttgtgtgtttctgcacgtttctgtgtctgtttgtctgtgtctctgtaggttctgcatgtccaaaaaagaatacagacgaagaggccaacaacaagggtggacatattgcagcaaacatgaaaaacaaagaattgctaccttatacataaaatgttcataatattagaaaacaaacacattaaggctccaagaataaaacaggcaagaagcagggtcagaaagttctcagaagagaagatacatttagtatacaagcatagaaaacgtccagtcttagaacttatatcaatgcaaatgaaagcaagtagatacatagttatataagaagaacaaaggttgagaggttgtgaatgctgttgttgttgaagcgagtgaaacaggtgctctcccatagcccgcaaactcgtatagtcctgttggaaagcattttgctgcatttgacccagtaattatacttgtggcataaatcctaaagaaatcattccataagctaaaaagcaaacttttaagaagcatctatacagaagtagattaagtaagccttgataaatcactagattttggaatatctcagattttcctgacaatgggaatcacccaaagtacttaccatgtatgcaagttcctctccctgggaaattctgattctgtacctctgggatggtgcccaggaatctatattttaaaaaggcactttaggctattcttatcttcagacacatttggaaaatactgatagaggaaatataatgaaatgccatcatgaggtcattaaagctaatgtgtgcaaagatcgtataattcttttttttttttttttttttttcagacaaagtctcactgttgtcccccaggctggagtgcaatggcacgatctctgctcactgcaacttccaccttccgggttcaagcaattttcctgcctcagccttcccagtagctgggattacaggtgcccgctgccatgccaggctactttttgtattttaagtagagacagggtttcaccatgttggccaggctggtgtcgaactcctgacctcaggtgatccgcccgccttggcctcccaaagtgctgggattacaggcgtgagcaaccatgcctggctgcaaagatcatataattctatggaaaaatacttaatgacattttgagttcctagaatgtcaaatgaaatagcagaatataaaagtctgtgaagtattggtctattcaacaaataaatatttactgagcacctactaagggccagccaggtcgtggggagacagaagagaacaaaacagctgccatttatcctcatggagcttcgagtctaatgggaagataaagagtaaagttaagaaaacacacacacacacacacacacacacacacacaaaattccatacttacctaactgcatggccatgatctctttacaaacacattgtctccttccatgggcggagagctgctgcagaaccaactgcttttggtgggattctagctccattacttagcaagtgcttgcaactctgtagcagcttaggaaagaactgtggttggaaggaaagagtgtggtgcatggatttggtaaaagagtaaaaagagtggctgggcacggtggctcatgcctgtaatcccagcactttgggaggccgaggcgggcagatcacgaggtcagcagtttgagaccagcctaaccaacatggtgaaaccccgtctcttctaaaaatacaaaaattagccaggcatggtggcacacgcctgtagtcccagctacttgggaggctgaggcgggagaattgcttgaacctgggaggtgaaggttgcagtgagcagagattgcaccactgcattccagcctgggcgacagagtgagactccatctagaaaaaataaaaataataaaagaaaaaagtaagaagagtaggagcagaaagaaagtgagttaataaatgaccagggctgtttctgaattctgtatggtggggcagaaaagattttctttaagtagacttctgggtacctgtagacagacgtgctgaaaacccactggcagaacagcagccctggtctggagggaccatgttggtctccagaagctaataccacaggtcagagttcagatcacccaccccaaatctgggatctgggatcagtatgagtctaggactggggcaaaagcccggggtggggatagagggctgtgtgaattgacctgccattcagaaacagcctcaagtttaggcttggagttatctccaaatgagattatgaatactgtcacagagagccacccgtaagatcgaaaaaaaaaaaaattaaccaggacttttacacttgtgtgttatgactgagctgtattgactctgatgcagtctgaatattttaaaaataaatcatacgcttatctgggaaccaaaaaaatatgttgcattatagttggttgaagtaaatatttaatatcctggatatgatagtttttataattctgggttggcatttcttccttgtatcaaaaactatactaaggccagttgcagtggcttgtgcctgtaatcccagcactttgggagcctgaggtgggcggatcacctaaggtcaggagttcaagacaagcctggccaacatggtgaaaccccgactccactaaaagtacaaaattagccaggcatggtcgcgtatacctgtaatcccagctacacgggaggctgaagcaggagaatcgcttgaacctgggaggcggaggttgcagtgagcggagatcatgtcattgcactccagcctgggcaaaaagagcgaaactccgtctcaaaaaacaaacaagtaactatattagaatcctcaaacgctggaagtggtttaagcctgccctgactctgagaggctattccagggtaagaatgctgcccagtactctcaaaccctgtagaaaaggggctggtgcttatttccttagaggcatttctgtgtagtttatctttggtgctaatgcggtccttttcaacttaccgtgttaaacaggacattagggttctgttaagaagagatgcactttgggaggccgaggcgggcggatcacggggtcaggagattgagaccatggtgaaaccccgtctctactaaaaaaaaatacaaaaaaattggtcgggcatggtggcgggtgcctgtagtcccagctactccggaggctgagacaggagaatggcgtgaacccaggaggcggagcttgcagtgagccgatatcacgccactgcactccagcctgggcaacagagcaaaaaaaaaaaaaaaaaaaaaaaaaaagatgtcgctgagtgagggagaacctctcctgggatatgtcctaccaggaagcatatctgcaggatcagattacacagattacaggaggtaacagagctggggacttagaaacagcagctgtctagtttcctatttatttactcattctgagcactgtccattggaatttttttaggaaggcaggtttggtgtgggctaggtagttgagatcctgagacctgctggtcttgatctgtagggagctgactggatgaccttggccccaggcctgccatagatgtaacagggaagatgcacttggccatctccaagggccactgcagcccagaacattctacgttaataagactcaagagtgtttgcccaatggcaaaaacaaaagtcacaccttccaactcagaccatccaaacggtttatgaacttccaagttttatttgttgaatcccacaggtctatcatcattgtaaactcttattccccccagtaatatatctgtaataatcctgaagcatgaatatcttgaaaatagctgcagatgcctatattttcccagcagagccgataaaagagacttttgtttacatattcatcattcagagtgctttgagaaattaggaagtaaatcgagttgcaattctgcaagtgacttggcccttaggactgtcttacagtgtgtggtgtgtaccttgtgcctattcaggaccattcctatcaaaatgaatttgtaatacaaacatgtcttcagccaatgggaccacagaatctcaccttgtcataagagatgcaatcagaagtattgtgcaaacacctttccctgacagaataagttcctggcaacccagtagccccctgcataatcaaacagtaagccagatcctaaatgttctatataaatgtagaatatggaaactgtagtcaaacaaaaatagcaatagtggggtagaaaccaggactctgtacttctgtatttcagtccttgtgtccttcagtccttctcaggccacgtttagtttgttttaacaacctcagcctagaactgcccttaattctggcaacaagggccctcctctggccccatgctttcaaggatctgctctcctgcaggtgtggctcctttcttagggggaaatgccgggctaaggaatgtatccctcaaggcctgggcctccctattttagaacattctctggatacccaggattccccgctcaaatgttctgggcctatttctaggacctgcccaggttctttgcttggtccatcctcctgagggcagactatactgaagccttaggctaaagaaggggcagcttttttgtggggagacggccagcagaacttggacctgtgggccgagatgtgcacccaggtgcatgtgaggactttctcagtgcaagatggagctggagggagtgggatgggaaaggaggtggtatcatgtgctggcagctggctctccccatgccaacgtgttccgggaaaaaattccaaggagcctgagaactcttaacttggatctagtcttctaggtcataaatgaaggtgtgcatatatatcaaggtagaaggatatgttatctttaaaagttttgttagtttcagccaggcatggtggctcacgcctgtaattccagcacttcgggaggccaaggtgggcagattacctgaggtcaggagttcgagaccagcctggccaaaatggtaaaaccccatctctactaaaaaaaaatacaaaataattagctgggtgtggtgacgggcacctgtaattccagctacttgggaggctgaggcaggagaatctcttgagcccgggaggcagaggttgcagtgagctgagatcacgtcactgcactccagcctgggtgatagagcaagactccatttcaaaaaaaaaaaaaaaggtttgttagtttgattggtaatgtttaaatatttagacatggagtaggtgggtctcccacttgtgatcttgttctgagtgaaaatgttaggggctgagctgccttaagcaaatctcttcacctctgaggcttggagctcctctgtaccaggaagccttgggctccttgagggctactggccggtccagctctttctttctttgaatgttggctgatgaggctgaaactgatgaagaaaaatgtaggcaacttctttccatggctgctttaggtgggattcttttcagtgcaagggacaacaatctaactcaaatcaccttaagcaaaagagagattctttctgttcacttgcttcagacatgttcatatttagttactcaaacaccatgttgtccataatttattcctatttcttcttctgttttcgttttttgagatggagtcttgctctgtcacccaggctggagtgcagtggcaggatctcggctcagagcaacctctgcctccagggttcaagcaattctcctgcctcagcctcctcctgagtagctgggactacaggcatgcaccaccaagcccagctaatttttgtatcttcagtagagatagggtttcaccatgttggctaggctggtcttgaactcctaacctcaagggatccacccacctcagcctcccaaagtgctgtgattacaggcgtgagccaccatgcccggcccctatttcttgactcagctttttttctctattggcttcattttggggcaagccaagatggccacaagcacctccaagcttgaatttggcaacttcagcaaaagagaacattcctttcctaataggttcagcaaaaatcctaactaagcctctcattggccctggctgggttacatgctcatcctctaaacaaatcactgtgactcaactgccaggaagctgggggagtggaagacggcggactcgcctgaaccacagggcagtgtggggcaaagggtatttccaacaggaaaagaggggttctgatgctggaagaaggatgctatgtaggcaaaatcaacagatgtttcaccagcaatgcttaccacatgaactatgaggacaaaggaaacagaaacatacaaatatttatgaaagacagcgatgaaatggtgcggtggaaaattgtgctagagaagccaatcctgccccctcaacgcagccacactgagcgagctgtgggtcaggggtacccaccctaccctctccttggctccaaagcagatgttcactacagtcaacttagacattgtgactcagagactgcaagttctgtcagacacttggactgaggatctacatggagataagcagagaaaggtggtctgtgagagaataaagcggaaatgcaaagaacaccagagaccaggcagccccagatagaccaagagctatgactccttccctccagccagtggctccagtgccttgcaaggctcagctgtatttcctgcccttggtagagactcctgggtccctccaacatgttttcgcgcgcgtgtgtgtgtgtgtgtgtgtgtgtgtgtgttacagctggatttaacagtttgctgttccacaaaccacaaataaaacaaaacacaataaaaacataaaggtggggaaatgctgttttttcttctaacatgtaagaattgagtcaggtgtttctcaagactgttgtgatttttatcttagtttttcacaaacatccagagaagggatagggaagcgtgcacgtggaacgacaaggcggctgagttcaaggtctggagcaagaagctctgcatccctgcagctctgatggggacggagaccctctgggcagagatatgcagggaaatgctcattactctgtaccccctaccccaacaccgcttttgccaagaggtggactgtgctagcaccaatgtggagagttttggacatccacgccatatctgtagcagctgcggctatctcaatgcataagctacattctcaaagaatttcacgtcaaaccagtgtttataaacggagcccgattttcagtgcttggagagaacctacacgcttccgttaaaatctctcttctagaaaagtgaaacacaacctgttaatcagcatttatataaggcaatattttaaaaatcagaaaaaagctttttttaaaaaaggcaaagttgacaagacaaataagctggatgaatcaaatttctgctttgttctgctttcactaattgctgacagagccgagttgcggcctgattataaagctgtgcttcagccaccttagcaaatctgttgctggaagacaaggagcgagcacttactttttgagagtaaactgtattttattttttattatactttaagttttagggtacatgtgcacaacgtgcaggttagttacatatgtatacgtgtgccattttaaaagcaccgggggactggtctatttaaaagaacaatggggtgagtggcgctctaatgacggactccagcttgggggctttgactatcctagttcttcttgggccccttttggctgagcgtgaagcaaataaacaaacaccccgatggagaggtccttaaccacggtgtgcagcagcatcacctggggagctgtagcccagtacacacgcccagccccacccaccagccttactgagaggggaagggatcctgcctgtgtgagctggaaaagctctccaggtgattccgcttcaagcttccggttaagcacgaaggctaatgagccttatttaaaagctcaggtttttactcagcaaaatctgttgcttttaaaatggaccgcctttagaaaaaccagcaatgttgcatgccaggatgggactctctccccggaaatgaaataagcaacccctgagaaacggcgctgggacaatagggcagcagtttctcctcacgtcctaggagggaaagtcgactgcagggagttatatgacttaatatgcagctaaccagccttttaattaacttgacatgccagataacaaagctattactaagtgagagtttcttaattgaaagggggaagagagatttgttttatattttcaaaataatctataatgagcgttactaatttgacaatcagaatttgtgtgtgtgtgaaaaatagctattttgagctatgaaaagggaggatgagcagacctgcacacggcagcttagcttgctgtggttttgccttagctggtagacggtgcctggtagtgcatgactgaaagatggtgtggttgattctattagtgtgcaattgttcgcaggcattttacctagaaatcacttgtgccatcgtggccatagtatttttccagcctcatctcttactgaactgtacctctagctctgagtccagtcacaatgaactaatttgtagtctctcagtcatccatgctttgcacatgcagtttcctctctatggaatatgaaatacctccccttccctcctcttccttcccttcagcttccagactcctgccagcaagcttataagtcacctttcaaatctcagttcaaaagcctcctctgagaccatctctccacttgcaagactcgggggctccatctatctcctgggatccctcgaccaggcactctagactgtcattatagcaactcattgagtgtattacgatggtgtgcttttgtgcctgtctccccaccattcatatagtcaacacgcacttggtagatgtcatcatttgatcactgcagcaatcctacagggtaccttttactgtgactcccatttcccagtggaagaaactgaggctcaaacatagtagcctgcccagctctcactacaagtagatggtttacgtgtgatacaatccaggttcatcttgcttctgagtttgtgctcttaactgccatgtgagcaaacttcaatcagaaagtgttttttcttttttcttttctttttttttttttttttttgtgacagagttgctctgttgcccaggctggagtgcaatggcacaatctctgctcactgcacctccacctcccaggttcaaacgattctcctgcctcagcctcccgagtagctgggactacaggcgcccaccaccacacccagctaatttttgtatttttagtagaggtggggtttcaccatgttggccaggctggtctcgaactcttgacctcaaatgatccaccttggcctcccaaagtgctggaattacaggcgtgagccaccgcaccctgcctgagagagactgtcttttcgaatttgtatcttcaatgcccagcctacaggagatgctcagtggataatgatggataattatttagcagttatccattgccaaaagaatggataacatcactgctaccggctttggcagacctcactccaggtaaatcattccctgggggcattaattacctgctggtgttccctggttaaaacacctgtgacaccagcctacacatacgcacagggctctgaggtgattttttttttaatgacaataaagacataaaaagatataaggtaaacctacgtgggctgcttatagcactgtcagttatgtgtgtgttttcatttacttcaaaaactgaggatattaaaataaatatgactttattccatttagttgagattgtcatttttttttaatttggaagagaatttaagaaatgatgactttattaacaacattggcgtaggacagtagcagactgggttaaaatactgtatcaatgttgaatttactaaagttcatcactgtagtacagttttggaagagaatatctccattctcagaaaatgcacactgaagaatttaggggtaaagggctataatgcacacaactgactcggatgtctcagaaaataagtgtgtgtgcatgtgtgtggtttgtatgtacgtctgtgtatgaggaagtgaaagggactaatgttaacaatagatgaatctgtgtgaaaaataaatgcatattctggctgggcacagtagctcacacctgtaatcccagcactttgggaggttgaggcaggcggatcacttgaggtcaggcgtttgggaccagcctggccaacacagtgaaaccctgtctctactaaaaaaaaaaaaaaaaggctgggtgtggtgacatgcgcctgtagtcccagctacttgggaggctgaggcaggagaatcacttgaacccaggaagtggaggttgcagtgagccgaggtcgctccactgcactccagcctgggcaacagagaaagactccacctcaaaaacaaaacgaacaaagaatggatgcgtattcttcatattattcttatttttgcaaattttctgcaagtttgaaattatgtccaaacgaccttggaagaaatgaacatccctgagaggaaggtgtaatgagagtgtttctttgaaatacagtgagcaagagctggcagggccggtcagtgtctgacagtggcatgaggtttctttcaggctgacttgcaatggctggttttctttacctattgatgtgtcttgaatatgtttacagttcagctggcccagttctctgagaggcaattgggtttccttgcagatgtgccgcgggaaggacagtggtgcctgtgcttggagaagcccctggccacgtgctaggacagagggacatatggtggcacgactccagccacagatgcaactccctcaggaacagtggggcctgcagttggaaggggccccctctggctcacagtgctgtgtggacagtagcatctgtgtgactgcaaactcgcccactgtgagtgggaacagtcgaggctatctgtggccttgcatctgctggtcccattcaccagggcaacactgtgcatggccaattctagacctcccggacgcagtgcatgcaactcagcgttagaatgtcaatttcgaagtactagaatgtcattttgctgttacagtcaccccacaagcattttctgagcatcttctacttgggattgcatcctttttgctagggactgtgtcatgtgcgtacacacagcatcttatttttagctttcaggctgacttgattgaacatggtgcagttaatgtgccccccattttccaaaagtagaaaactgtgacacagaggttaagtggtttctgaggtaacatagaaaaaatatgtagcagagatttcctaaacaaacttgcagcctggcaggaggggtaagaagatccacgaggaacattggatcaggttggaggaaagaggtgccaagagagacccaagatcttggctgggaagtgaaaaggagtgtggccacttttgattctggggtaggaggctttattggggaggtggcatttgcgtggagactaacaggatgataagaattttgaaaggaaaatcataaagagctttccaatggagtcgagaaaacatggtaaaaaaacaaaataggagttgagatcataacaactgtcatttattgagtttttctatatgctaggaactgtgagaggcgctttagataaatcaactcattgaaacaggagttttcttaagtgagccctattagcatcctcattttagggtaaatggaggcatccatggaaggttacatgcatctagtgtggtaacaaagcccacaagcttagaaagtgcttcatgataatagtgaaatgatggtaataataggaaaaaggagggggaggaggagggagaggggaagaggaagaggaagaggagtggggaggaggagaggaaaaggagaaggagaggaggggagggggaggaggaagaagcagcaggaggaagagtggaaggagaaggggaagaagaaggaggggcaaggggggaggaggatgagaagaagggagaggagaaggagggggaggagaagggggaagggggagaaaacaagagggaggagggggaggaggagaaggagggaggtaggaggaggagtgggggacaaggagggaaaggagaaggggaagagggagaggatgaggagggggaggtggaggaatgaggagggagaggaagagagaggagaggaaggagaagggggaagggagagtagagaaaggaagaggagggaggagagggaagaggagggaggagagggaagaggaggaaacgagaagaggggagaagaggagggaggagttggggaggaggaaggggagaagggagaggagagggaggaggaggaatgaaaataggcagggggaggaggagaagagggaggatgggagaagaggtaggagggggaggagagggtggagtggggttaggggttagtcctggaggcatcagaggcttctctagggagcgtggtttctatcctactctaccttagccttgaccaagcaggcagatagcattagtattcactccttgcttgggagcacttgaaaagtttataaaaaggcgtaggctgtttggataaaagatgctctggagacaagacagtgcatcttcctcagtcacttcctcactcctttctcggctctgattctggtgtttgatgtcttcccacaactcggcaaagaaagaagaaaatccctctactcactgtgcagtttgtaggttatttaaaggaaatgcattcaggtggttccttacccggcagggtgcagggatggagtgggatacaaccatacaaccaacccctcagagggcaagcgcagctcattcacagtggccaggatccctagggcagcctcgggcgtctgtcccgcagcagaggacactctcatgaggcgctggaaactcagctcagggcgtgccaggtcccacgggcgccttccagcctgggacacctgtgccaaacctgaacagggaaggtgcagaaaagcgtgtgtgtgcgcatgcacgtgtgtgtgctaaaatataaatgaacgattaagggtttcctctgctggatattctctgcagtggggagaagaggtgggagaaagtagctgtttttgccgcttggggaatgtttgcccaactggtaaaggtagaattgttcttttccaaaggaaagttgtgtgggagttgcttccttaccgaaaacaaggaaaagcattagtgaaaagatgtaagatcaacaggcaatcaaaaatgcacactgccagtgttaagggcacaggtgaattttccttctaggattctcaatacaaacctattttgaaataaaatgcctctaggtcttccctgcctaaacccacgtggggagcactaatagctgcgtacaaacttcattaaactggccacagctgaaaggagctggtgccaacccactgctttttgctgaccgaagtatccggctgggtttttgccctcattctgaagtgactgctgcccatcccccacaccttgagcattgttttactagacatcttctagtgtagggtaactggaagaaaagtaatggaataccaagtgccattcatcatatccctgcctcttctattttgtggtgcagggatgctgaggggaaaatgagtctcctgtaagtgcttggagatcctcccccactccacctcctgcatttccataagcatttggcatcagagtcttctggtaaaccccccagcttctacaattggacaattggctttgtatcacggcaggaattcgtgcctctgaagtttctagggaagctctacagaagcaataaagtggtagagttgtttgaataaaattagcttctatgcttgtaggaagcatacccaattccagttagctgtatgaaatgcaaccattttggaggtttgtgaaaatatgcaaggctcccggcttcaggagaaaaacagatttacattcctccctgtctcagcagggagtcttcaatcaaaggcaaccaacaaatcaaacatgattatctgtcagcacattggccctggtttgtaattatacatttatttgtgtgtgatcaatgctagtctcctcactggattctaaactccctgagagcttttctgtcttaattaccctgaactccagtgcccacacagtacctggcacatagctcatgctgtaaatatctgtggaaagaaggaagaaatggagaaaaggaagggaggaaggaacagaagggagaaaggaaaacggaaaaaaagaaatgttccaggtggaaggatttttttttttttttacaatcatcctgcccaacagtatataggtttgcctgtgatctttttctcatacataagatggagataatagtccttgtctcaatagttattttacgttattttctaactcaaatagttaaaagtcatttgtaggcccctgctctgggcccatgctttgtaggatctcactgtcgctgtcctcaggctgtgccccttcctagagtatgaagtcccggtgggactttaagcctatgctccccttccccttcctccgcatctgtggggacttctccccgacagttcacgcaggtctccaccacaagtgtgcatgccctaggcccaaggggtgtccaaggagtgactatttgtaggggatgagccatggatggaactgtggtgtctgcacacatgtgcctaagaccctctcccattgtgggatggagcctgcagttcagtagggggaatgaagggaggtgtgaatcatggctcttgacccaggcccgcctctctctgtgtggccagggttcagggcagaacctcaggaggctggaagttgtagcttctaacctggcctttcaggtcatgatgaaggtctatttgtcagggtaagaggttcaaacctcctgcaatagtcctattcagcagctgatagcttggtttataacttttgaatatttagatgtattccacgtgggcaaataggaacacacacacatatatatgtatatttgtgcatttatatgtgtgggcatgtgtgtgcacgtgtgtgtacatatataattctatagttcacctgttagtgtaccttgatgatgaaaagtgagggaggaccctgactttggacagcatggatctgcctgccacttaccagctaaactgtttccttagggcaaaaatagagacaacaatagtacctatttagttggattattgacattattaaaagagagcaactaacatactcctagaatataagtgctccatgcatattataaactaacaattgtttcctgctcctttcacttcatgcatgaagacatattcactcactcataaatacttgcattatatctatctatctatctatctatctatctatctatctatctatcatctatcaacaaagtcttgttctgttgcccaggctagagtgcagtggtgtgatcctagctcactgtagcctcgaactcctgtgctcaagcaattctcccacttcagcctcctgagtagctgggactacagatgtgcaccaccatgcctggctaatttttgcatttatttgtagagatgagctctcactatgtcgcccaggctggtctcgaactcctgggctcaagtgatccttctgcctcggcctcccaaagtgctgggattaggagtgtgagccaccatactcggccattatgtatatttcttattcaatctgagaactaactataatattattcatttactattttagttcaagttgatttccttttaaaacatacacaccaagtttatgtgtattgataccagtggtttcccaggtgtttttttgttgttgttttgttttttcagattctcattctgttgctggagtgcagtggcgctatcttggctcactgcaacctctgcctcccgggttcaagcgattctcctgcctcagcctcccgagtagctgggactacagacacgtgccaccacgcccagctaatttttgtatctgtagtagagatggggtttcaccatgttggccaggatggtctcgatctcttgacctcatgatccacccgccttggcctcccaaagtgctgggattacagacgtgagccaccatgcctggccttatataggtatttcacaaaatgatttcctctattaggaccatattcaaaaagcccttcccctactccacaattacagaagcagtcacatacattccatttgattcttctctatgatttcatttttgaaacttaattccttaacccacctggaatttattgcggtgttgttgtgaggttaagaaaaaaaaaaatcaatctaatataatgtttctaaaaagccagttgtctcggcatcatttttggaataatctttcccctcatcattcatttacatttctacctttgtcacatagttaatactttttttcaatttgggtttctttctaaacctgtaagtcaattttaatgatctagttaacttttgatgccagtatataccgttttaattcttgcaggtgcataacagttaatacagcagagcgcaagggctgcttagttttcttgtttttcccttttattttgggtgggttggggaagggaacaaggtcttgctctgttgcccaggctggagtgcagcagcgtgatcacagctcaccacagcctcaacctcttgggctcaagccatcttcccacctcagcctcctgagtagctgtgattacaggggtgcgccaccatgaccagctaattttttttttttttttttgtaaagacagtggtcttgctttgttgcctaggctggtctcgaactcctgggctcaaacccacctcagcctcccagagtgctagaattacaaacatgagccactgtgcctggccatttttcttctttttcaaagttgatcaattatgtgagcatcaccactagaatctgcaaatgtctcctgtatcggcaacgagggaggtaccataagcacccttcttttacagatgaggaaactgagcacagaaagaagagacacttgctcaaggtcacaaaaacaaggcaggtccaggaacagtgaaacacaggcagtctagctgcagggaccacgatcataacctctgcaaagtggggcagatccaacctgagaatcaatctccttcaagtcggagcattttctcctcatatctattattactgacttcttagtatttgttttatttatttggttgtttaatgatttcatatgtttccctgtgtttcgttatatactttctatttataatgcttcttaaagttttctggttacagactattttctttctttttttctgagatgtggaacttaccatggttcatattttaaactctttggctaggtttactaataattgtgcttacccgaaagcattctttaactgctatttctttggttttcaaggtcagtgactctttatatggctgcatacacattttagtacaatgataactggataattttaataaagttgtataagatatagtttacgaacataaaaatgattctattattagctaaaatttcagcagcactgttgacataatttttattgttttaattaaattgcatggaaaagaaataattttatcataagaataaagaggatgatagttcaaagttatttgtgagaatatcgtggctgtattgcattagcatcttgacttttaaggtgatgtttaatagagacacaacaattctttaggtcgtaaaggcaattcttgctgttttaaaaaaatgttatgacaacaggtgtgatcacataaagtattagtaaagatgaaacaattttaaatattttccactctatattctactgctttataagaaggctgacaagaaaaccctcatttcactagatcatatctacatctcactggcaggaaagaagggcccatatgagttacttacctaagtaggaactattattcctgttttacagatgagaaaaccaaagctcagaggctaagtgactagttgaatgtcagcagaccaattgaagaaaactcaaaatgtcaccactcaccaaattcacctgtctatccagccagtgcacacatccttggcagatgtctcctaattaagtggagtgtgtgtgtgtttgtgtgtgtgtgtgtgtgcgcgcgcgcgcgcgtgcgcgcgcagtgaggtgggccaccccgcctgcaggcagctctaagtcatagttccgttaattatttattttatatgatgattttgagtccttttgtagtcctggctgtctttttatgagcacatttctatttgagaaagtcagcaggaatctggattctggaatcactgaattccaatgctagctccaattcttcctagaaacgtgatcttagaaacgttaatttatataacagaaatgataatacatatcttacaggtatggtgtgagagttaaatgagaagttgtccatgtatttagcattgtgcctgactggtatcatgtgctaatgcatactgctcattttattttatttccatggtatggacgtccttttaagaatattcgcccactgtagctgggcgcggtggctcacgcctgtaatcccagcactttgggaggccgaggcaggcggatcacgaggtcaggagatggagaccatcctggctaacacagtgaaaccccatctctactaaaaaaaaaaaattacaaaaacttagctgggcatggtggcgggcacctgtagtcccagctactcgggaggctgaggcaggagaatggcgtgaacccgggaggcggagcttgcagtgagacgagatcgcgccactgcactccagcctgggcgacagagggagactgtctcaaaaaaaaaaaaaaaaaaaaggatattcgcccagtggaacaactttggctgctggtccctcctctgtctcccccaagcagggttatatagttcgttgagacattcccttcaccaaaaggcattcctcagctcagggaaaggaaagtggagaggaatggtgagtgagaccgtctttaaatatcctgaactactgcccccttccttattgtctactatctacatttggggagtgattctcttagcaacctctcaggtttgatatcagcaatactgactcatgatactaccccaaagccaaagcatgaaacatggaaggtgttcactagggacaataccagatttccttaaatcacaaagcaacagagcacatcacactggatgtctcactctggcttcctgcccggctccatatcaacgggcaattgacgttggggggagccatttcctactctggccttcagcttgcggtcagctgagtgtgttggaccacacactctctagcatcctgcgattctaaccttctatggatttcatcagttttatagatatgagttcagcctacgactttgggaaacaaaggattcaactgtaaaaaacatttgaattccactgatctattttatctctgctcaggaagaaaaaatggcaccttcttcctgaagtttgtgtttccggtctccttgatttctgagagattttaaaattactttctatttttcttactctgttctgatattgcaaaatggttattaccaattattaactaagtgatgtttaattttagaagtcaagctacttgtaagggcccatataaatgtgtgctaggattagctttagatttgttttctgcttctatttacagcaaggacaggactggggagtggttttattttattaagctttttagcatgatttaatttttaaaactcaggacgtattactttaaaaattaatcgaataaagatgtatgttcataacttgaaccacacagaaaagtaaaatacaaataaaattgtgatctcattacttaaagaataaccattgttggccatgtgcggtggctcacgcctgtaatctcagcactttgggaggccaaggcgggcgcatcacttgaggtcaggagttcaagaccagcctggccaacgtggtgcaacctcatctctactaaaatacaaaaaaaattagctgggcatggtggcgtgtgcctgcaatcccagctacttgggaggctgagccaggagaattgcttaaacccgggaggccgaggttgcagtgagcagagattgcgccactgcactccagcctgggcgacagagcaagactccatcacaaggaaaagaaaacaagcattgttaaaattttgatgcaattccttgtagcctactcattcactgtttctaatgcttactaagtgtttagtaacacatacatacacactgcacacacacacattgtctccttcttcactcaacataaggatagcatttcctatattattaaaatatttttaaaaatgtgtgtgtgttacatgtgttatatgtcacacacacttttaaccacacaaagacacaggagaacatcaaaaatcaagatgctttcacgtcccctcacacatgtgatccttataatcctgtgtgagaagcaggactggaaatatttccaacttccagctgaaaatgcatagctcagagacaggaaggaacttaacgttggttaagatcacaggctcggggtaccacataccagctgtgtgaccctgggcacaataatggatctaagatttgtggggcgcgaagcctgtatcattttaggggttctccttaaagaaaataataaaacatttacctgtgaaaattttagtgatttcatgtgatcttgtaagtatattgctaggacctcttccagggccttggaagggtctgtgttaagtgaggagccctgtagcttcatttcatctgcttggaggcaaatctgcctttatttgggtaagtgacttattttcatctgtaaagtggggataataaaagtgcttgcctctgagtagttagaaagattaaacaagatactgtattgtaaagcattttgtaaacttcctggcacattggcacataataagtgcttaataagggtcacctgtgattactaattttattcaaaatcatgtcattgtggctggtgtcatttgagctgcttcccagagactgagcgattcctgtacatacctaaagttacaccttcaagatgctgcagcttggctcactcactcatttaataagcatttaggagttcctgctagatgctatgcactgtgctaggctccagtctcaattcattctcacaccacattcactggaagcacaactcaggtatcccctcctctgggaagcccttctaggaccctaagccgactcactactatctgggcacttatctctctgtgtgactgggtttggacatcactagtattcaaggaaaagacattatcctgcccctctgccacctttgttcatttcagttcagtataatcgatacttctctctgtgcctataatacagtatggaggtgctcaataatcttaaatgagttgactgagcatgtgtttgttttcacaggaagatttccgtttcttttgcaagctatttaatttgcaaaagtaagcaagatgtgcacaaaatagttttgagacatctggaaacaaaacaaggttgcctcatcattaatcttgtttttgtgtgataactttactttttctcattttatgacaactgaaattctctattatactgccagacctcattctgcaagcttctctcctgtgctaataaaaaatattatggccacatcgagaagtccttagggaatgtgttctgcatcaggaaaagtaattaagctctggggtcctaaaggagcctgggaaagtctatccagaaactatggggttaggatgtattatctattgaaaaacagaaccggactttgcaagttttacaatatcttggcttattaaagccactaactgagaattaaaatttctggattgttacttttacaacagcagtcaagtgtcggaaaatatcctgaccagtcagtaaggtatacaaatagagaaggcaaggagtagctgtgagtaaagcgccaactacatttgctgagtacctgggaatttacgagttagcttttgctatcattatccgtctcgctaaagcaaccctatgaggtaggtgggaagctggatgccgtcctcttttgacagccaacactgaagaacagctggggctggaaactagatctgtcagacatagtaactgcttctatcactctcaccaccctcccatgctcttgagagtgccttcgcttttgtgggtgtcttcagaaaagcatgcggatctctgtataggttttactcaagtgttcctctctgtggagggtgacctgggctacatgaacatgggcacctcaggatcggcagctttccatgaattcctatggtaaggggttcagcttatccttcatgtgggtgaagatgtatgatttcattgaacattggcagttacagccaagtacaagtcctgccttcaggatccagcagggaagaatgacattaaacatgtcaccttggagaaatgttgcattcaccttccgggtaatgacccagccacccagggactcctctgaaatatccaatcctctaagtttaaacacgtttcagaattaatccatctgaattcttatcgctgtagatgcaaggagaaggagttatggcaggtctgaaactattagcggccaagctccctagcagaagcaacctctccctacaccccattatccgtgcacagctccttatcagcggaggaacaactttactgtcaccatattttctacttggaaaaaaaaaagaaacctcagcaggcccaatccgaaggctatgaaatttcaaagaaacagagctaagaggcgagaaactagccctttgtgttaaaaagatggaaatgctccaagcgcctttccagtctgctttctgtttacaggccttgcgtgagcgcgggaggctgggcctcatctctggctctccccagccaggaccccttactcaaaaccctccatctcggcaagaaccctcattcccaagttagttggattccaagtccataaaccgggtcaaaagaatacagtaatttcctactggagctctaagtggtggttttcacggaggactcggcaccatcctcccacctgcctcctcccatcgaacattcctttttaagaaaaacacacaccaggctccgggaagctgacgtaaacatcctgaggaaataaccactgtaagtggcttctaaacccatttccccaaggaaataatcagcacctctttcccaagacagctccaggtaagcaagcggtgaagggagctgcaccaccgcgttctcaaaagtaaaggcgcttgcggaactgtctactgatttgtaagcgcgcgcccatccactgtcgcatttaatcttccgaacgacccacgaggtggtaaaggcggggattattttcttcattttacgggtgagaaaccgaggcccacagcgctcgttcctgtagccggggtcaggcagggcacacctaggggagcctctgccttcgagccccgggaccgccccgcggcaccacgagatctccccagtcagcccgtgtgcggctgcggccgcatggcctcattgttttgggaagacgtccctctgtgaggatcttgggcgactctatgaaccgcgggcccagccgctctgcggaacgatccgcagcgggacgcaaagggcgcggcgagcccggcggctcccggaacaaaggacagcagagcgcgcggggcccgaaggggcgtccgccctagtgggcggcggagggggatgcgcgcggagaggaccagcgcgcaccgccccggcccgcccctcaaatcctccttccttctctctcgcactcggagacggtccctgggagatccgggagggggcgcagctcgccgtcctcgccggcaagtgccgtcgcaacctccctctgccgccacccccaccccgagaagcgcacaaagagcggccgggcagggagcgctcacctcccgtcggggcggggccgcgggcggggccggcgcgcgctccgcagcgcccgccttaaagggcccgcccgctcctcgcgcgcactgcgcatgctcggccgcggggcacggaggggagggatgggaacagcgggcgcgcacgcccgcgccgcccgctggcgctgtggcctgcgtccccgcggtggcggcgcggcgctcgtgcgcgtgtcagaacccgcagggtctcggcccgggcgccgggcgtgtgctggacactggtgccatgcattccagaggtcgccagcggccgggcgggccgagctcgcgcggcagccagcttttagctttcccatcctcagtttcagggccagttgggcgaagtgctgcccaaggagacagaaatgcaggcgcgggcgcgcgcgcgcgcggttgccagtgtgggcgggcgtgtgcttttgtgtctcgtgcgctcccgcgcaggtggacaacccgcgccgggagtcactctgcccgtgcgccccaagacctggagtcccgttttccgtgtcggagggctcgggtcgcccttttgggcggactacagactcttctcacagaggaagctttggctccacggatggtttatttggagccactaacgggacttcctgaggaccgctcttttagagcccggctccaggcatcagagttgggcgcgttttcttttctcagtcaggcgagggaggagacttagggacaatgattgtcctcggctgataggtacatccaagtgtcccgagcctgccagtcccgcattagacaacaaagagaggcgttagcggcggcgggggaggggcgcggccgggaggaggacggggcgggctgcggcgagcgcgggggtggggggtggcgctctctctccgctcgctcaacccgcggcctcctcccgcccccggcctggcgcgcgccaatcgcctcccccagcgatagtgtcagtagcattgtggtgtcagctcccgcctgtgacgttgcgcctccctcgtccccctccggagtcgtctggctgcagaggctc

SEQ ID NO: 3 - DNA, 836 bp, Human
gtaggtcgaggagggatggggaggtgggtgggggtggtgtagggtctcaggccactgcctcgaggggaaggcgtgttcagtatcgggatccgcggcgtggggtgccttggggagagaggaagagccgcgcgatgggccggcgccccagacaaagaaagtgcaggcaggctgtctcccggagccgcgccgctgccctggcgggatgcactttcttctgctaaaatcactgccttctcccctaacgccccccaaccagcccacctccagaaagacaatttaaatgtaagatgcttgggggagggggcctttgatcagtcctttgggaggaggaaggaggaggagtgagcataggatgggaggaggattctggatttctgcaaagcggaatggagcccagaggaggaacaatgggtcccgggactcacaccccaccccctacccccagtcgaccagcgctgaggcatcgcgacttcagctgccttccccgagccccttccccgtgtcttcagagctgacggcgcgcccagctggatcccagcggcatctccccagatgacttttctgggattctcgggtttggttcgggacgactgcagtcactgggggagggccaggcagccaatgggctgttcctcgagcgcctcgcgggtgggatccgctgcccagcccgtggcgcggcccgaggtcagtgagggagacgccccctttccgcccatctcttgtcctgccgtctcgctgtcctggacgcgggctgtccccggtccccgcggttaccccaggataatgggcgtgtctgtctctctctcccactccctcctccgcaccctggttcgtag

SEQ ID NO: 4 - DNA, 3416 bp, Mouse
tgttcgctttgcgctcggcattgtggccagccagccgggcactcggggggcacgcgcggccgccgctcgagctctgcccccaccccaaccgccagcagatctggggtggggacccaggcgggggctcttgcagccactgcccggtgcggattgcacgcagagacccactcctccgagcgccgaaaaacgagccacggagccctccgcagccgaccggcctccccgcccctgactgccggcttcccggctgcctttgtggctgcaccttctagctgccgagcagagagccggctggggcgcggcgcgcacggcggagcgatgcccagctcgctgtttgcagacctggagcgcaacggcagcggcggcggcgggggaggcggcggcgggggaggcggcggtggcagcggcgggggagagactctggatgaccaaagagccctgcagcttgcgctcgatcagctctccctgttgggactggacagtgatgagggcgcctctttgtacgacagcgaaccgcgcaagaagagcgtgaacatgaccgagtgcgtgccggtacccagttccgaacacgtcgcggagatcgtagggaggcaaggttgtaaaatcaaagctttgagggcgaagaccaacacttacatcaagaccccagttcgcggggaggagcctgtctttgttgtgacgggcaggaaggaggatgtggctatggctcggagggagatcatctctgccgcagagcacttctccatgatccgagcctctcgtaacaagaacacggctctcaacggagctgtgcccggaccgcccaacctgccgggacagaccactatccaagtgagggtgccataccgcgtggtagggctcgtggtgggtccaaagggcgccacgatcaagcgcattcaacagcagacacatacatatattgtgacacccagccgagacaaggagccagttttcgaggtgactggcatgccagagaacgtggatcgcgctagagaggagatcgaagctcacatcgcgctgcgcaccggtggcatcatcgagctgacagacgagaacgacttccatgccaatggcacagacgtgggctttgatctgcatcacgggtccggcgggtccgggccgggcagcctctggagcaagcccaccccaagcatcactcctacacctggccgcaagcccttctccagctatcgcaacgacagctccagctcgcttggcagcgcatccacagactcttacttcggtggtgggaccagcggcagcgcagctgctacttcacgcctggcggactatagccctcccagccctgcactcagctttgctcacaatgggaacaacaacaataacggcaatggttacacctacacagcgggggaagcctcagtaccttccccagatgggggtcctgagctgcagcctactttcgacccagctcccgccccaccacctgggacaccccttctctgggcccagttcgagcgctctccaggaggtggatctgcagcaccagtatcctcttcctgctcttcttcggcatcctcatctgcctcgtcgtcctctgtggtctttcccgggggtggcgccagcagcacaccctccaatgccaatctggggctgctggtgcaccgtcgactgcacccgggcaccagctgcccgcgcctgtctccgcccttgcacatggccacgggggcgggagagcaccaccttgctcgccgcgtgcgcagcgacccgggcggtggaggcctggcctacgctgcctatgctaatgggctagggacgcagctccctggcctgccctcgtcggacacttcgggctcctcctcgtcctctagctcctcctccagctcttcctcctcttcctctgggctgaggcgcaaaggcagccgcgactgctctgtgtgcttcgagagtgaagtgatcgccgcgctggtgccctgtggccacaacctcttctgcatggagtgtgccaaccgcatttgtgagaagagcgagcccgagtgtcccgtctgccacacggcggtcactcaggccatccgcattttttcctgaaggcagtgcgcgcgcgcgcactgcagggaaggagggtcctctctcgaccctcattccctagggtctacctgcccagacgcctctggtgcccacctctttccaccccaccctcatcactctcagagatcccagaggagcttggaaagctgtagtatccgctcatttttaaaatgtcatttttaaacaaaggaacttgccaggatctctgcatcaggagtactgtagcctccgaaccacctgaattgcatgctctataaataataggaacggcgacattctagtaacgatagtttttacactgtacttaataggaagcttccaaaagaaaaccccacaagttttccattttcttgaagtagaaaaatgaacagtaattatgaagatgattaataattgtgctatgggatgtgtggactgttttgtgtgtttccctttgtgggtgggttcctacagcgctcgttctagaacacaagtggatcctttttgaatgttcatggaagggccaggagttctgtacagccaggaccctgcagctttattaaagttaaaactgtaacatatctcttatatattaaaaaaaaaaacctttaaaagttttaaagagaaattgcattaatacagattgaagtattttattctttttttgacttgaaaaattatatttcatattgcaaagatgtttacaagtattttaatttaagttcagtgaacttttttgtagctgggttaaatctttttatttttagtatggccttatggcaaagaacactgtattattttaataatcacacgattgtgacggattacaaaccataaaatgtataacgttttgagcagtattctgttgggatggagattttataggttcagacaaatcttctagatctgcttcacccagcatattttctattcagtgatataaagcatattttattctatattattacaaaaaatggaaatgtataaacatgtcaaaaggaacagttgatgctttctaacatttgtataaatagaattcagtgcaaattacagaaattctgttgcaccgctatagttttagtgtttctattttaatacatttgtttaccactcgtttatgtatatgtaggtgacgttacttgagcttaaatgtactttactgagcaaagtttaaaaaaaaacaaagtatattttattttatgataaagggcctttaacctcatggtcaaatactaatattatatttgctgagacaagatttgaaattgtatcaagagttttatttttctgacatttaaagttctacataataaaggtaaacttaagtaatggtgctacttcattttttaagtatttctatataaataaaacattgaagaaaaatcact

SEQ ID NO: 5 - protein, 569 aa, Human
MPSSLFADLERNGSGGGGGGSSGGGETLDDQRALQLALDQLSLLGLDSDEGASLYDSEPRKKSVNMTECVPVPSSEHVAEIVGRQGCKIKALRAKTNTYIKTPVRGEEPVFVVTGRKEDVAMARREIISAAEHFSMIRASRNKNTALNGAVPGPPNLPGQTTIQVRVPYRVVGLVVGPKGATIKRIQQQTHTYIVTPSRDKEPVFEVTGMPENVDRAREEIEAHIALRTGGIIELTDENDFHANGTDVGFDLHHGSGGSGPGSLWSKPTPSITPTPGRKPFSSYRNDSSSSLGSASTDSYFGGGTSSSAAATQRLADYSPPSPALSFAHNGNNNNNGNGYTYTAGGEASVPSPDGCPELQPTFDPAPAPPPGAPLIWAQFERSPGGGPAAPVSSSCSSSASSSASSSSVVFPGGGASAPSNANLGLLVHRRLHPGTSCPRLSPPLHMAPGAGEHHLARRVRSDPGGGGLAYAAYANGLGAQLPGLQPSDTSGSSSSSSSSSSSSSSSSGLRRKGSRDCSVCFESEVIAALVPCGHNLFCMECANRICEKSEPECPVCHTAVTQAIRIFS

SEQ ID NO: 6 - protein, 576 aa, Mouse
MPSSLFADLERNGSGGGGGGGGGGGGGGSGGGETLDDQRALQLALDQLSLLGLDSDEGASLYDSEPRKKSVNMTECVPVPSSEHVAEIVGRQGCKIKALRAKTNTYIKTPVRGEEPVFVVTGRKEDVAMARREIISAAEHFSMIRASRNKNTALNGAVPGPPNLPGQTTIQVRVPYRVVGLVVGPKGATIKRIQQQTHTYIVTPSRDKEPVFEVTGMPENVDRAREEIEAHIALRTGGIIELTDENDFHANGTDVGFDLHHGSGGSGPGSLWSKPTPSITPTPGRKPFSSYRNDSSSSLGSASTDSYFGGGTSGSAAATSRLADYSPPSPALSFAHNGNNNNNGNGYTYTAGEASVPSPDGGPELQPTFDPAPAPPPGTPLLWAQFERSPGGGSAAPVSSSCSSSASSSASSSSVVFPGGGASSTPSNANLGLLVHRRLHPGTSCPRLSPPLHMATGAGEHHLARRVRSDPGGGGLAYAAYANGLGTQLPGLPSSDTSGSSSSSSSSSSSSSSSSGLRRKGSRDCSVCFESEVIAALVPCGHNLFCMECANRICEKSEPECPVCHTAVTQAIRIFS

SEQ ID NO: 7 - DNA, 4368 bp, Human
tcaagaggcggggaggagaggaggaaaaagcgctgagtgagggcgggcgggcgggcgggagggagggagtggaggagccggggaggggctccttaaagaaacgcttctgtcgctcgcctgctcgcttttcgctcggcattgcggccagccagccgggcactcggggggcacgcgcggccaccgctagagctctgcccccaccccacccgccagcaggtctggggtggggacccaggtgggggctcctgcagccactgcccggtgcggaccgcacggagcgacccactcctcccagcaccgaggaagaagcaacggagccctcagcaggcgaccggcctccccgcccctgaccacccgcttcccggctgcctttgtggccgcagcttctcgccgccgagccgagggccggcgggggcgcggcgcgcacggccgagcgatgcccagctcgctgttcgcagacctggagcgcaacggcagcggcggcggcggcggcggcagcagcggagggggagagaccctggatgaccaaagagccctgcagctcgcgctcgaccagctctccctgctggggctggacagtgacgagggcgcctctctgtacgacagcgagccgcgcaagaagagcgtgaacatgaccgagtgcgtgccagtacccagttctgagcatgtcgccgagatcgtggggcggcaaggtaggtcgaggagggatggggaggtgggtgggggtggtgtagggtctcaggccactgcctcgaggggaaggcgtgttcagtatcgggatccgcggcgtggggtgccttggggagagaggaagagccgcgcgatgggccggcgccccagacaaagaaagtgcaggcaggctgtctcccggagccgcgccgctgccctggcgggatgcactttcttctgctaaaatcactgccttctcccctaacgccccccaaccagcccacctccagaaagacaatttaaatgtaagatgcttgggggagggggcctttgatcagtcctttgggaggaggaaggaggaggagtgagcataggatgggaggaggattctggatttctgcaaagcggaatggagcccagaggaggaacaatgggtcccgggactcacaccccaccccctacccccagtcgaccagcgctgaggcatcgcgacttcagctgccttccccgagccccttccccgtgtcttcagagctgacggcgcgcccagctggatcccagcggcatctccccagatgacttttctgggattctcgggtttggttcgggacgactgcagtcactgggggagggccaggcagccaatgggctgttcctcgagcgcctcgcgggtgggatccgctgcccagcccgtggcgcggcccgaggtcagtgagggagacgccccctttccgcccatctcttgtcctgccgtctcgctgtcctggacgcgggctgtccccggtccccgcggttaccccaggataatgggcgtgtctgtctctctctcccactccctcctccgcaccctggttcgtaggttgtaaaatcaaagcgctgcgggcgaagaccaatacttacatcaagaccccagttcgcggggaggagcctgtctttgttgtgacgggcaggaaggaggatgtggccatggctcggagggagatcatctctgctgccgagcacttctccatgatccgcgcctcccggaataagaacacggcactcaacggcgcggtgcctgggccgcccaacctgcccgggcagaccaccatccaagtgcgggtaccctaccgcgtggtggggctcgtggtggggcccaaaggcgccacaatcaagcgcatccagcagcagacgcacacgtacatcgtgacgcccagccgggataaggagccggtgttcgaggtgaccggcatgccagagaacgtggatcgcgctcgagaggagattgaggcgcacattgctctgcgtaccggcggcatcattgagctcacagacgagaacgacttccacgccaacggcaccgatgtgggcttcgatctgcatcatgggtccggcgggtccggcccaggcagcctctggagcaagcccacccccagcatcacgcccacccccggccgcaagcctttctctagctaccgcaacgacagctccagctcgcttggcagtgcttccacagactcttatttcggcggcgggaccagcagcagcgcagcggctacccagcgcctggcggactacagcccccctagccccgccctgagctttgcgcacaacggaaacaataacaataacggcaatgggtacacctacacagcggggggagaagcctcagtgccatcccccgacggctgccccgagctgcagcccacttttgacccggctcccgctcccccacctggggcaccacttatctgggcccagttcgagcggtccccgggaggcggacctgcagctccggtatcttcttcctgctcttcttctgcatcttcgtctgcttcttcctcctccgtggtcttccccgggggtggcgccagtgcgccctccaacgccaacctggggctattggtgcaccgccggctgcaccctggcaccagctgcccgcgcctgtctccacccttgcacatggccccgggggcgggagagcaccacctggctcgccgggtgcgcagcgacccgggtggaggaggcctggcctacgccgcttatgccaacgggctgggggcacagctgcctggcttgcagccgtcggacacgtcgggctcctcctcttcgtccagctcctcctccagctcttcatcctcttcctccgggcttcggcgtaaaggcagccgcgactgctccgtgtgcttcgagagcgaagtgattgccgcgctggtgccctgtggccacaacctcttctgcatggagtgcgccaatcgcatctgtgagaagagcgagcccgagtgcccggtctgccacaccgcggtcactcaggccatccgcatcttttcttaaaggcagcgggcgctgctagtgcgcaccgtgctgggggaagggggaacccctccccaccctctttccccagcgctcgcctgcctccctgggtgccccccctctcccttctccttcccggccccaccaacactctgagatccgagaggagcttggaaagctgtagtatccgctcatttttaaaatttaatttttaagtaaaggaatttgccaggatatctgcatcaagagtactgtagcctgggaaacctgaacacctgaaatgcatgctctataaataataggaacggcgacattctagtaatgatagtttttacactgtacttaataggaagcttccaaaagaagaaaaccccacaagttttccattttcttaaagtaggaaaaaatgaacagtaataattatgatgaagatgatagtagtgctatgggatgtgtggactgtttagtgtgttcccctttgtgggtgggttcctatgatacttattatagaacacagtggatcctttttgaatgttcgtggaagggccaggagttcctgtgaaaccaggatactgcagctttattaaagttaaagaaactgtaacatatctcttatatattaaaaacgtttaaaagttttaaagagaaattgcattaatacagattgaagtattttattcttttttgacttgaaaaattatatttcatattgcaaagatgtttacaagtattttaatttaagttcagtgaacttttttgtagctgggttaaatctttttattttagtatggccttatggcaaagaacactgtattattttaataatcacacaattgtgacggaattacaaccataaaatgtgtaatgttttgaacagtattctgttgggatggagattttataggttcagacaaatcttctagatctgcttcacccagcatattttctattcagtgatataaagcatattttattctatattattacaaaaacggaaatgtataaacatgtcaaaaagaactgttgatgctttctaacatttgtataaatagaattcagtgcaagttacaaaaattctgttgcaccactctagttttagtatttctattttaatacatttgtttaccacttgtttatgtatatgtaggtgatgttacttgagcttaaatgtactttactgagcaaagtttaaaaaacaaagtatattttattttatgataaagggcctttaacctcatggtcaaatactaatattatatttgctgagacaagatttgaaattgtatcaagagttttatttttctgacatttaaagttctacataataaaggtaaaacttaagtaatggtgctacttcattttttaagtatttctatataaataaaatattgaagaaaatcttaaaaa

SEQ ID NO: 8 - DNA, 16 bp, Artificial Sequence
  hmrGD-89
gagcggatactacagc

SEQ ID NO: 9 - DNA, 16 bp, Artificial Sequence
  hmrGD-89-2
gcggatactacagctt

SEQ ID NO: 10 - DNA, 15 bp, Artificial Sequence
  control
aacacgtctatacgc